European Patent Application EP 4 123 305 A1, published January 25, 2023. Title: A prefabricated microparticle for performing a detection of an analyte. Applicant: Blink AG. The sequence listing filed with the application follows.

SEQUENCE LISTING (6 sequences)

SEQ ID NO: 1 - DNA, 19 bp, synthetic construct
  source 1..19: mol_type = other DNA
  misc_feature 1..19: note = sense primer
gcagtggcgcccgaacagg

SEQ ID NO: 2 - DNA, 22 bp, synthetic construct
  source 1..22: mol_type = other DNA
  misc_feature 1..22: note = antisense primer 1
actgacgctctcgcacccatct

SEQ ID NO: 3 - DNA, 23 bp, synthetic construct
  source 1..23: mol_type = other DNA
  misc_feature 1..23: note = antisense primer 2
tgacgctctcgcacccatctctc

SEQ ID NO: 4 - DNA, 125 bp, synthetic construct
  source 1..125: mol_type = other DNA
  misc_feature 1..125: note = oligonucleotide for labelling detection antibody
gcgtcagaccccgtagaaaagatcaaaggatcttcttgagatcctttttttctgcgcgtaatctgctgcttgcaaacaaaaaaaccaccgctaccagcggtggtttgtttgccggatcaagagct

SEQ ID NO: 5 - DNA, 20 bp, synthetic construct
  source 1..20: mol_type = other DNA
  misc_feature 1..20: note = forward primer for PCR in embodiment 3
agctcttgatccggcaaaca

SEQ ID NO: 6 - DNA, 20 bp, synthetic construct
  misc_feature 1..20: note = reverse primer for PCR in embodiment 3
  source 1..20: mol_type = other DNA
gcgtcagaccccgtagaaaa